European Patent Application EP 4 810 615 A1, published September 23, 2026. Title: Microorganism and a method for producing L-arginine using the same. Applicant: CJ CheilJedang Corporation. Application KR. The sequence listing filed with the application follows.

SEQUENCE LISTING (80 sequences)

SEQ ID NO: 1 - protein, 259 aa, synthetic construct
MSNFETFLWVAYPWLCIAAYIIGISWRWRADQFGWTTHSSQIYESKLLRIASPLFHWGMVFVVIGHLMGLAIPKSWTQAVGISDAAYHLIATIPGTIAGIAAVLGLIGLIVRRVINKTVFLSTSRSDKVMYVLLGAAILSGFIATVSTQVFGGAHGYDYRETISPWLRQLLIFNAQPELMADVPWEFKVHIVAGFTLIALWPFTRLVHAFSAPVGYVTRPYVVYRTRDTTSEPARQNVAWEPIRSVKNQLDNDSKWHGA

SEQ ID NO: 2 - DNA, 780 bp, synthetic construct
  source 1..780: mol_type = other DNA
atgtcaaactttgaaacgttcctctgggttgcctacccctggctgtgtatcgccgcctacatcatcggcatttcctggcgctggcgcgccgaccaattcggttggaccacccactcctcccaaatctacgaatccaaactcctccgcatcgcctccccactcttccactggggcatggtgttcgtggtgatcggccacctcatgggacttgccatccccaagagctggacccaagctgtaggaatttctgacgccgcttaccacctcatcgccaccatcccaggcaccattgccggcatcgctgcagtccttggactcatcggtttgattgtgcgccgagtaatcaacaagaccgtcttcctgtccacctcacgctccgacaaagtgatgtatgtgctactcggcgctgcaattttgtcaggattcatcgccaccgtctccacccaggtcttcggcggcgcacacggctacgactaccgcgaaaccatctccccatggctgcgccaactgctcatcttcaacgctcaaccagagctcatggctgatgtcccttgggaattcaaggtccacatcgtcgctggattcaccctcatcgcactgtggccattcacccgcctagtccacgcgttctccgcaccagttggatacgtcacccgcccctacgtggtctatcgcacccgcgacaccacctctgaaccggcacgccaaaacgtcgcctgggaaccgatccgctcggtcaaaaatcagctcgacaatgactcgaaatggcacggcgcctaa

SEQ ID NO: 3 - protein, 477 aa, synthetic construct
MAFETPEEIVKFIKDENVEFVDVRFTDLPGTEQHFSIPAASFDADTVEEGLAFDGSSIRGFTTIDESDMNLLPDLGTATLDPFRKAKTLNVKFFVHDPFTREAFSRDPRNVARKAEQYLASTGIADTCNFGAEAEFYLFDSVRYSTEMNSGFYEVDTEEGWWNRGKETNLDGTPNLGAKNRVKGGYFPVAPYDQTVDVRDDMVRNLAASGFALERFHHEVGGGQQEINYRFNTMLHAADDIQTFKYIIKNTARLHGKAATFMPKPLAGDNGSGMHAHQSLWKDGKPLFHDESGYAGLSDIARYYIGGILHHAGAVLAFTNATLNSYHRLVPGFEAPINLVYSQRNRSAAVRIPITGSNPKAKRIEFRAPDPSGNPYLGFAAMMMAGLDGIKNRIEPHAPVDKDLYELPPEEAASIPQAPTSLEASLKALQEDTDFLTESDVFTEDLIEAYIQYKYDNEISPVRLRPTPQEFELYFDC

SEQ ID NO: 4 - DNA, 1434 bp, synthetic construct
  source 1..1434: mol_type = other DNA
gtggcgtttgaaaccccggaagaaattgtcaagttcatcaaggatgaaaacgtcgagttcgttgacgttcgattcaccgaccttcccggcaccgagcagcacttcagcatcccagctgccagcttcgatgcagatacagtcgaagaaggtctcgcattcgacggatcctcgatccgtggcttcaccacgatcgacgaatctgacatgaatctcctgccagacctcggaacggccacccttgatccattccgcaaggcaaagaccctgaacgttaagttcttcgttcacgatcctttcacccgcgaggcattctcccgcgacccacgcaacgtagcacgcaaggcagagcagtacctggcatccaccggcattgcagacacctgcaacttcggcgccgaggctgagttctacctcttcgactccgttcgctactccaccgagatgaactccggcttctacgaagtagataccgaagaaggctggtggaaccgtggcaaggaaaccaacctcgacggaaccccaaacctgggcgcaaagaaccgcgtcaagggtggctacttcccagtagcaccatacgaccaaaccgttgacgtgcgcgatgacatggttcgcaacctcgcagcttccggcttcgctcttgagcgtttccaccacgaagtcggtggcggacagcaggaaatcaactaccgcttcaacaccatgctccacgcggcagatgatatccagaccttcaagtacatcatcaagaacaccgctcgcctccacggcaaggctgcaaccttcatgcctaagccactggctggcgacaacggttccggcatgcacgctcaccagtccctctggaaggacggcaagccactcttccacgatgagtccggctacgcaggcctgtccgacatcgcccgctactacatcggcggcatcctgcaccacgcaggcgctgttctggcgttcaccaacgcaaccctgaactcctaccaccgtctggttccaggcttcgaggctccaatcaacctggtgtactcacagcgcaaccgttccgctgctgtccgtatcccaatcaccggatccaacccaaaggcaaagcgcatcgaattccgcgctccagacccatcaggcaacccatacctgggcttcgcagcgatgatgatggccggcctcgacggcatcaagaaccgcatcgagccacacgctccagtggacaaggacctctacgaactgccaccagaggaagctgcatccattccacaggcaccaacctccctggaagcatccctgaaggcactgcaggaagacaccgacttcctcaccgagtctgacgtcttcaccgaggatctcatcgaggcgtacatccagtacaagtacgacaacgagatctccccagttcgcctgcgcccaaccccgcaggaattcgaattgtacttcgactgctaa

SEQ ID NO: 5 - DNA, 1434 bp, synthetic construct
  source 1..1434: mol_type = other DNA
atggcgtttgaaaccccggaagaaattgtcaagttcatcaaggatgaaaacgtcgagttcgttgacgttcgattcaccgaccttcccggcaccgagcagcacttcagcatcccagctgccagcttcgatgcagatacagtcgaagaaggtctcgcattcgacggatcctcgatccgtggcttcaccacgatcgacgaatctgacatgaatctcctgccagacctcggaacggccacccttgatccattccgcaaggcaaagaccctgaacgttaagttcttcgttcacgatcctttcacccgcgaggcattctcccgcgacccacgcaacgtagcacgcaaggcagagcagtacctggcatccaccggcattgcagacacctgcaacttcggcgccgaggctgagttctacctcttcgactccgttcgctactccaccgagatgaactccggcttctacgaagtagataccgaagaaggctggtggaaccgtggcaaggaaaccaacctcgacggaaccccaaacctgggcgcaaagaaccgcgtcaagggtggctacttcccagtagcaccatacgaccaaaccgttgacgtgcgcgatgacatggttcgcaacctcgcagcttccggcttcgctcttgagcgtttccaccacgaagtcggtggcggacagcaggaaatcaactaccgcttcaacaccatgctccacgcggcagatgatatccagaccttcaagtacatcatcaagaacaccgctcgcctccacggcaaggctgcaaccttcatgcctaagccactggctggcgacaacggttccggcatgcacgctcaccagtccctctggaaggacggcaagccactcttccacgatgagtccggctacgcaggcctgtccgacatcgcccgctactacatcggcggcatcctgcaccacgcaggcgctgttctggcgttcaccaacgcaaccctgaactcctaccaccgtctggttccaggcttcgaggctccaatcaacctggtgtactcacagcgcaaccgttccgctgctgtccgtatcccaatcaccggatccaacccaaaggcaaagcgcatcgaattccgcgctccagacccatcaggcaacccatacctgggcttcgcagcgatgatgatggccggcctcgacggcatcaagaaccgcatcgagccacacgctccagtggacaaggacctctacgaactgccaccagaggaagctgcatccattccacaggcaccaacctccctggaagcatccctgaaggcactgcaggaagacaccgacttcctcaccgagtctgacgtcttcaccgaggatctcatcgaggcgtacatccagtacaagtacgacaacgagatctccccagttcgcctgcgcccaaccccgcaggaattcgaattgtacttcgactgctaa

SEQ ID NO: 6 - DNA, 42 bp, synthetic construct
  source 1..42: mol_type = other DNA
gtgaattcgagctcggtacccatggcaattgaactgaacgtc

SEQ ID NO: 7 - DNA, 42 bp, synthetic construct
  source 1..42: mol_type = other DNA
cagagcgagcccgacagtactttgctgcactaataaggcccc

SEQ ID NO: 8 - DNA, 42 bp, synthetic construct
  source 1..42: mol_type = other DNA
gccttattagtgcagcaaagtactgtcgggctcgctctggtg

SEQ ID NO: 9 - DNA, 42 bp, synthetic construct
  source 1..42: mol_type = other DNA
ggtcgactctagaggatccccatgtcaaactttgaaacgttc

SEQ ID NO: 10 - DNA, 18 bp, synthetic construct
  source 1..18: mol_type = other DNA
ctccgaatgggtaaaccg

SEQ ID NO: 11 - DNA, 18 bp, synthetic construct
  source 1..18: mol_type = other DNA
cctaaattcctcacaagc

SEQ ID NO: 12 - protein, 171 aa, synthetic construct
MSLGSTPSTPENLNPVTRTARQALILQILDKQKVTSQVQLSELLLDEGIDITQATLSRDLDELGARKVRPDGGRAYYAVGPVDSIAREDLRGPSEKLRRMLDELLVSTDHSGNIAMLRTPPGAAQYLASFIDRVGLKEVVGTIAGDDTVFVLARDPLTGKELGELLSGRTT

SEQ ID NO: 13 - DNA, 516 bp, synthetic construct
  source 1..516: mol_type = other DNA
atgtcccttggctcaaccccgtcaacaccggaaaacttaaatcccgtgactcgcactgcacgccaagctctcattttgcagattttggacaaacaaaaagtcaccagccaggtacaactgtctgaattgctgctggatgaaggcatcgatatcacccaggccaccttgtcccgagatctcgatgaactcggtgcacgcaaggttcgccccgatgggggacgcgcctactacgcggtcggcccagtagatagcatcgcccgcgaagatctccggggtccgtcggagaagctgcgccgcatgcttgatgaactgctggtttctacagatcattccggcaacatcgcgatgctgcgcaccccgccgggagctgcccagtacctggcaagtttcatcgatagggtggggctgaaagaagtcgttggcaccatcgctggcgatgacaccgttttcgttctcgcccgtgatccgctcacaggtaaagaactaggtgaattactcagcgggcgcaccacttaa

SEQ ID NO: 14 - protein, 317 aa, synthetic construct
MNDLIKDLGSEVRANVLAEALPWLQHFRDKIVVVKYGGNAMVDDDLKAAFAADMVFLRTVGAKPVVVHGGGPQISEMLNRVGLQGEFKGGFRVTTPEVMDIVRMVLFGQVGRDLVGLINSHGPYAVGTSGEDAGLFTAQKRMVNIDGVPTDIGLVGDIINVDASSLMDIIEAGRIPVVSTIAPGEDGQIYNINADTAAGALAAAIGAERLLVLTNVEGLYTDWPDKSSLVSKIKATELEAILPGLDSGMIPKMESCLNAVRGGVSAAHVIDGRIAHSVLLELLTMGGIGTMVLPDVFDRENYPEGTVFRKDDKDGEL

SEQ ID NO: 15 - DNA, 954 bp, synthetic construct
  source 1..954: mol_type = other DNA
atgaatgacttgatcaaagatttaggctctgaggtgcgcgcaaatgtcctcgctgaggcgttgccatggttgcagcatttccgcgacaagattgttgtcgtgaaatatggcggaaacgccatggtggatgatgatctcaaggctgcttttgctgccgacgtggtcttcttgcgcaccgtgggcgcaaaaccagtggtggtgcacggtggtggacctcagatttctgagatgctaaaccgtgtgggtctccagggcgagttcaagggtggtttccgtgtgaccactcctgaggtcatggacattgtgcgcatggtgctctttggtcaggtcggtcgcgatttagttggtttgatcaactctcatggcccttacgctgtgggaacctccggtgaggatgccggcctgtttaccgcgcagaagcgcatggtcaacatcgatggcgtacccactgatattggtttggtcggagacatcattaatgtcgatgcctcttccttgatggatatcatcgaggccggtcgcattcctgtggtctctacgattgctccaggcgaagacggccagatttacaacatcaacgccgataccgcagcgggtgctttggctgcagcgattggtgcagaacgcctgctggttctcaccaatgtggaaggtctgtacaccgattggcctgataagagctcactggtgtccaagatcaaggccaccgagctggaggccattcttccgggacttgattccggcatgattccaaagatggagtcttgcttgaatgcggtgcgtgggggagtaagcgctgctcatgtcattgacggccgcatcgcgcactcggtgttgctggagcttttgaccatgggtggaattggcacgatggtgctgccggatgtttttgatcgggagaattatccggaaggcaccgtttttagaaaagacgacaaggatggggaactgtaa

SEQ ID NO: 16 - DNA, 40 bp, synthetic construct
  source 1..40: mol_type = other DNA
tgaattcgagctcggtaccccactggtgaactccttgtcc

SEQ ID NO: 17 - DNA, 40 bp, synthetic construct
  source 1..40: mol_type = other DNA
ttgaactaggggcgctttaaaagttttccggtgttgacgg

SEQ ID NO: 18 - DNA, 40 bp, synthetic construct
  source 1..40: mol_type = other DNA
ccgtcaacaccggaaaacttttaaagcgcccctagttcaa

SEQ ID NO: 19 - DNA, 40 bp, synthetic construct
  source 1..40: mol_type = other DNA
gtcgactctagaggatcccccgttgaactgcttgccagcc

SEQ ID NO: 20 - DNA, 40 bp, synthetic construct
  source 1..40: mol_type = other DNA
tgaattcgagctcggtaccctgcggctcgcacggttgctc

SEQ ID NO: 21 - DNA, 40 bp, synthetic construct
  source 1..40: mol_type = other DNA
acggtgcgcaagaagaccacgtcggcagcaaaagcagcct

SEQ ID NO: 22 - DNA, 40 bp, synthetic construct
  source 1..40: mol_type = other DNA
ggctgcttttgctgccgacgtggtcttcttgcgcaccgtg

SEQ ID NO: 23 - DNA, 40 bp, synthetic construct
  source 1..40: mol_type = other DNA
gtcgactctagaggatccccctcttatcaggccaatcggt

SEQ ID NO: 24 - protein, 357 aa, synthetic construct
MIMHNVYGVTMTIKVAIAGASGYAGGEILRLLLGHPAYASGELEIGALTAASTAGSTLGELMPHIPQLADRVIQDTTAETLAGHDVVFLGLPHGFSAEIALQLGPDVTVIDCAADFRLQNAADWEKFYGSEHQGTWPYGIPEIPGHREALRGAKRVAVPGCFPTGATLALLPAVQAGLIEPDVSVVSITGVSGAGKKASVALLGSETMGSLKAYNTSGKHRHTPEIAQNLGEVSDKPVKVSFTPVLAPLPRGILTTATAPLKEGVTAEQARAVYEEFYAQETFVHVLPEGAQPQTQAVLGSNMCHVQVEIDEEAGKVLVTSAIDNLTKGTAGAAVQCMNLSVGFDEAAGLPQVGVAP

SEQ ID NO: 25 - DNA, 1074 bp, synthetic construct
  source 1..1074: mol_type = other DNA
atgataatgcataacgtgtatggtgtaactatgacaatcaaggttgcaatcgcaggagccagtggatatgccggcggagaaatccttcgtctccttttaggccatccagcttatgcatctggtgaactagaaatcggagcactcaccgcggcatcaaccgcaggcagcacgctcggtgaattgatgccacacattccgcagttggcggatcgtgttattcaagacaccacagctgaaactctagccggtcatgatgtcgtatttctaggacttccacacggattctctgcagaaattgcacttcagctcggaccagatgtcacagtgattgactgtgcagctgactttcgtctgcaaaatgctgcagattgggagaagttctacggctcagagcaccagggaacatggccttatggcattccagaaataccaggacaccgcgaggctcttcgtggtgctaagcgtgtagcagtgccaggatgtttcccaaccggtgcaaccttggctcttcttcctgcggttcaagcgggacttatcgagccagatgtttccgtagtgtccatcaccggcgtatcaggtgcaggtaagaaagcatctgttgcactacttggctcggaaaccatgggttcactcaaggcgtacaacacctccggaaagcaccgccacaccccggaaattgcccagaacctcggcgaagtcagcgacaagccagtcaaggtgagcttcaccccagtgcttgcaccgttacctcgcggaattctcaccactgcaaccgcacctttgaaagaaggcgttaccgcagagcaggctcgcgcagtatatgaagagttctatgcacaggaaaccttcgtgcatgttcttccagaaggtgcacagccacaaacccaagcagttcttggctccaacatgtgccacgtgcaggtagaaattgatgaggaagcaggcaaagtccttgttacctccgcaatcgataacctcaccaagggaactgccggcgccgctgttcagtgcatgaacttaagcgttggctttgatgaggcagcaggcctgccacaggtcggcgtcgcaccttaa

SEQ ID NO: 26 - DNA, 86 bp, synthetic construct
  source 1..86: mol_type = other DNA
caataatcgtgaattttggcagcaacagaattatgtggtataatggaaacgtgcaaaagcatagattattggaggagatcaaaaca

SEQ ID NO: 27 - DNA, 42 bp, synthetic construct
  source 1..42: mol_type = other DNA
gtgaattcgagctcggtacccgccccgaaaagccgttaaaag

SEQ ID NO: 28 - DNA, 42 bp, synthetic construct
  source 1..42: mol_type = other DNA
tgccaaaattcacgattattgcccacctacagctaaaactgc

SEQ ID NO: 29 - DNA, 42 bp, synthetic construct
  source 1..42: mol_type = other DNA
ttattggaggagatcaaaacaatgacaatcaaggttgcaatc

SEQ ID NO: 30 - DNA, 42 bp, synthetic construct
  source 1..42: mol_type = other DNA
ttaaggtgcgacgccgacctgggggatcctctagagtcgacc

SEQ ID NO: 31 - DNA, 21 bp, synthetic construct
  source 1..21: mol_type = other DNA
caataatcgtgaattttggca

SEQ ID NO: 32 - DNA, 21 bp, synthetic construct
  source 1..21: mol_type = other DNA
tgttttgatctcctccaataa

SEQ ID NO: 33 - protein, 445 aa, synthetic construct
MGSKYTRKDIVKLVEEENVRFIRLQFTDLLGIIKNVEIPVDQLGKALDNKMMFDGSSIEGFVRIEESDMYLYPDLDTFVVFPWTSEKGRVARLICDIYNPDGTPFAGDPRSVLKKVIQEMKDLGFTAFNIGPEPEFFLFKNDEKGEPTLELNDKGGYFDLAPTDLGENCRRDIVLELEDMGFEIEASHHEVAPGQHEIDFKYADAVKACDDIQTFKLVVKTIARKHGLHATFMPKPLFGVNGSGMHANMSLFKGEQNAFFDEKSDLQLSETAKQFIAGILKHAEAFTAITNPTVNSYKRLVPGYEAPCYVAWSSRNRSPLVRIPASRGLSTRIEVRSVDPAANPYLAMAVMLAAGLDGVKNNLTPPAPVDRNIYVMDKEERIENGIADLPATLAQALDTLKRDDIIMAALGEHAAEHFIEAKEIEWDMFRTQVHPWEREQYLTLY

SEQ ID NO: 34 - DNA, 1338 bp, synthetic construct
  source 1..1338: mol_type = other DNA
atgggttctaagtacacgagaaaagacatcgtaaagcttgttgaggaagagaacgtacgttttatacgtttgcagtttacagatttgctaggaattataaaaaacgttgagatccctgttgatcaattgggtaaagccttagacaacaaaatgatgtttgacggctcatccattgaagggtttgttcgtatcgaggaatcagacatgtatctctatccagatctagatacctttgttgtattcccatggacgagcgaaaaaggtcgcgtagctcgtttaatttgtgatatttacaatccggatggcacaccgttcgcaggtgatccaagaagcgtacttaaaaaagtcattcaagaaatgaaagatctcggctttactgcctttaatatcggaccagagcctgagtttttccttttcaaaaatgatgaaaaaggtgagcctacgcttgagttgaatgacaaaggcggctattttgacttagcaccaacggatctaggtgaaaattgtcgacgtgatatcgtgcttgagcttgaagacatgggctttgaaattgaagcatcacaccatgaagtcgctcctggtcaacacgaaatcgactttaaatatgcagacgctgtaaaagcgtgtgacgacattcaaacgtttaagcttgttgttaaaacaattgcacgtaagcacggcttgcatgcgacgtttatgccaaaaccattgtttggtgtgaatggttctggtatgcacgcaaacatgagcttgtttaaaggtgagcaaaacgcgttttttgacgaaaaatcagaccttcaattaagcgaaacagcaaagcaatttattgctggcattctgaagcatgctgaagcatttacagccattacgaacccaacagtaaactcatacaagcgtttagtgcctggctacgaagccccatgttacgttgcatggtcttctcgtaaccgttcaccactcgtacgtatcccagcttctcgtggcttgagcacacgtatcgaagtgcgttcggttgacccagctgcgaacccttacttggccatggctgtaatgcttgctgctggacttgacggtgtgaaaaacaacttaacaccaccagcaccagtagatcgcaacatctacgtgatggacaaggaagagcgtattgaaaacggcattgctgatcttccagcaacgcttgcccaagcgcttgacactcttaagcgtgacgatatcatcatggcagcacttggtgagcacgctgcagaacactttatcgaagcaaaagaaatcgaatgggacatgttccgcacacaagttcacccttgggagcgcgagcagtaccttaccctttactaa

SEQ ID NO: 35 - protein, 444 aa, synthetic construct
MAKYTREDIEKLVKEENVKYIRLQFTDILGTIKNVEIPVSQLGKALDNKVMFDGSSIEGFVRIEESDMYLYPDLNTFVIFPWTAEKGKVARFICDIYNPDGTPFEGDPRNNLKRILKEMEDLGFSDFNLGPEPEFFLFKLDEKGEPTLELNDKGGYFDLAPTDLGENCRRDIVLELEEMGFEIEASHHEVAPGQHEIDFKYAGAVRSCDDIQTFKLVVKTIARKHGLHATFMPKPLFGVNGSGMHCNLSLFKNGVNAFFDENADLQLSETAKHFIAGIVKHATSFTAVTNPTVNSYKRLVPGYEAPCYVAWSAQNRSPLIRIPASRGISTRVEVRSVDPAANPYLALSVLLAAGLDGIKNKLEAPAPIDRNIYVMSKEERMENGIVDLPATLAEALEEFKSNEVMVKALGEHLFEHFIEAKEIEWDMFRTQVHPWEREQYMSQY

SEQ ID NO: 36 - DNA, 1335 bp, synthetic construct
  source 1..1335: mol_type = other DNA
atggcaaagtacactagagaagatatcgaaaaattagtaaaagaagaaaacgtgaagtatatccgccttcaatttactgacattcttggaacaatcaagaatgttgagattcctgtaagccagcttggaaaagcgcttgataataaagtcatgtttgacggttcttctattgagggattcgttcgtatcgaagagtcagacatgtacctgtatccagatctaaatacatttgttatcttcccatggacagctgaaaaaggtaaagtagcacgtttcatctgtgatatttacaatccggatggcacaccttttgaaggtgacccgcgaaacaacttaaaacggattctgaaagaaatggaagacctcggcttcagtgattttaaccttgggcctgagcctgaattcttcttattcaaattggacgaaaaaggcgagccgacgcttgaactaaacgacaaaggcggatatttcgacttagctccaactgatttaggagaaaactgccgccgcgatatcgtacttgagcttgaagagatgggctttgaaatcgaagcgtctcaccacgaagtagcacctggtcagcacgaaatcgactttaaatatgctggagcagtccgctcttgtgatgacatccaaacatttaaactagttgtcaaaacaattgcccgtaaacacggcctgcatgcgacatttatgccaaaaccattgttcggtgtaaacggttcaggtatgcactgcaatctatcactcttcaaaaatggtgttaacgcattctttgacgaaaacgcagatcttcagttaagtgaaacagcgaagcacttcattgcaggtatcgtgaagcacgcaacaagctttacagcagtaacaaacccgacagtaaactcttacaaacgtcttgttcctggctatgaagcaccttgttatgtagcatggagcgcgcaaaacagaagcccgcttatccgtatcccggcttctcgcggcatcagcacacgtgttgaagtacgcagtgtagacccagctgcaaacccataccttgcacttagcgtattgcttgctgcaggattagacggaatcaaaaacaaactggaagcgccggctccaatcgaccgcaacatctatgtgatgagcaaagaagagcgcatggaaaacggaatcgttgaccttccagcaacacttgcggaagcactagaagaattcaaatcaaacgaagtcatggtcaaagcgctgggcgagcacctattcgaacacttcatcgaagcaaaagaaatcgaatgggatatgttccgcacgcaagtacatccttgggaacgcgaacagtatatgtctcagtattaa

SEQ ID NO: 37 - protein, 614 aa, synthetic construct
MSGGGCDTLFLKECPSMTSKEHPLTQEATRRVAGGERVIDVAEKLGIHPSTIYLALKRRGLPVGAGAPHRVLNPQTNRHIPNNPERPTTTEAVARVARGERVITVAKELGIHPSTIYLALKRRGLPVGAGAPHRVLNPQTNRHIPNNPERPTTTEAVARVARGERVITVAKELGIHPSTIYLALKRRGLPTSVPTPPADNDYGHHDQGTTPTPTTTVITSPGTTTQVPKTSDTTNELSSRTADDVTADFSLVPNTRIKTGRGVRLSSNDRLAIAQGIHEGLSTRAIGKKLGRHHSVIAREIARGSTRYTDPATTTVKKLVYNPQTAHYHAQQQARRPKVRILDHPSRLRDVVVEYLLRKFSPKRVEQRLQLDYPNDMSMHISHEAIYQSLYIQGRGSLREVIEEELRQRDMDPSKVLIRGGRSRKPRSKIAGLRNRRGWVVGAEITTRPPEADDRRVPGHWEGDLVIGAGGQSALLTLVERSSRFTLLKHLPDDHASSTVVGALQEMIASMPGKFSTITWDQGSEMASARKVIDPQVCGVYFCDPHSPWQRPTNENTNGEIRRRFYPKGTDFREVTAEHVAWVQDELNDTPRLVLGALTPYEKMNEVLTVATTQ

SEQ ID NO: 38 - DNA, 1845 bp, synthetic construct
  source 1..1845: mol_type = other DNA
atgtcaggcggtggatgcgacaccctcttcctaaaggagtgtccatccatgaccagcaaagaacaccccctcacccaggaggccacccgccgggtggccggcggtgaacgagtaatcgatgtagcagaaaaactcggaatccacccatccaccatctacctagcgctcaaacgccgtggcctaccagtcggggccggcgcacctcaccgtgttctgaacccacaaaccaaccgccatatccccaacaacccggaacgacccaccaccacagaagcagtcgcccgcgttgcccgtggtgaacgcgtaatcaccgtggcaaaagaactcggaatccatccatccaccatctacctagcgctcaaacgccgtggcctaccagtcggggccggcgcacctcaccgtgttctgaacccacaaaccaaccgccatatccccaacaacccggaacgacccaccaccaccgaagcagtcgcccgcgttgcccgtggtgaacgcgttatcaccgtggcaaaagaactcgggatccatccatcgacaatctacctagcgctcaaacgccgtggcctgcctaccagtgttcccacaccacctgctgacaacgactacggtcatcacgaccaaggcaccacacccaccccgacgactacggtgatcacatcaccgggtacaacaacacaggtgcctaaaacatcagatactactaatgagttgtcgtcgcggactgcggatgacgtcaccgcagattttagtcttgttcccaacacacggatcaaaaccggccgcggggtgcgcttaagcagcaacgatcgtttagctattgcccagggaatccatgagggactgtccactcgggcgatcgggaagaagcttggccgtcatcatagtgtcatcgcacgcgaaatcgcccggggttctacccgctacaccgatccggcaacgacaacggtgaaaaagttggtgtacaacccacagaccgcgcattatcatgcgcagcaacaggcacgccgcccgaaagtaaggatcttggatcacccaagccggttgcgggatgtggtggtggagtatttattacgaaagttttcccccaagcgtgttgaacaacgcctacagctggactatcccaatgatatgagcatgcatatttcccatgaggcgatctatcaaagcttgtatatccaaggacgcggcagcttgcgtgaggtcatcgaagaggaactgcgccaacgtgacatggatccaagcaaggtgttaatccgtggtgggcgtagtcgcaaacccaggtccaagattgctgggttacgtaatagacgtggctgggtggtgggtgccgaaattacgacacgtccaccagaagctgatgatcgtcgggttcctggtcactgggaaggtgatttagtcattggtgctgggggtcaatcagcgttgttaacgttggtggaacgctcaagtaggtttacgttgttaaagcatttgcctgatgatcatgcctcgtcaacggtggtgggtgcgttgcaggagatgattgcgtcgatgccggggaagttttccacgattacctgggatcagggatcggaaatggcgagtgctcgtaaagtgattgatccacaggtgtgtggggtgtatttctgtgatcctcattcaccgtggcaacgcccgacgaatgagaatacaaatggtgagatcaggcgccggttttatcctaagggcactgatttccgtgaggtgactgcggaacatgtggcctgggtacaagatgaacttaatgacacacccaggttggtgttaggtgcgttgaccccgtatgagaaaatgaatgaagtcttaactgtcgcaaccacccaatga

SEQ ID NO: 39 - DNA, 39 bp, synthetic construct
  source 1..39: mol_type = other DNA
aacgacggccagtgaattcgctcgaatgcctgactgaca

SEQ ID NO: 40 - DNA, 44 bp, synthetic construct
  source 1..44: mol_type = other DNA
gtttagtactaaaccggaagggccaaaggacgacttcacggtta

SEQ ID NO: 41 - DNA, 46 bp, synthetic construct
  source 1..46: mol_type = other DNA
ccggtttagtactaaacaggaagagccattgaggatgcgaaactgt

SEQ ID NO: 42 - DNA, 39 bp, synthetic construct
  source 1..39: mol_type = other DNA
tgcatgcctgcaggtcgacgtaatcgaatcaccggccag

SEQ ID NO: 43 - DNA, 20 bp, synthetic construct
  source 1..20: mol_type = other DNA
acgtgtgctgacttctcatg

SEQ ID NO: 44 - DNA, 20 bp, synthetic construct
  source 1..20: mol_type = other DNA
ctcattagtgcaaaggtatc

SEQ ID NO: 45 - DNA, 386 bp, synthetic construct
  source 1..386: mol_type = other DNA
ggcccttccggtttagtactgctccttagggagccatcttttggggtgcggagcgcgatccggtgtctgaccacggtgccccatgcgattgttaatgccgatgctagggcgaaaagcacggcgagcagattgctttgcacttgattcagggtagttgactaaagagttgctcgcgaagtagcacctgtcacttttgtctcaaatattaaatcgaatatcaatatatggtctgtttattggaacgcgtcccagtggctgagacgcatccgctaaagccccaggaaccctgtgcagaaagaaaacactcctctggctaggtagacacagtttattgtggtagagttgagcgggtaactgtcagcacgtagatcgaaaggtgcacacat

SEQ ID NO: 46 - DNA, 44 bp, synthetic construct
  source 1..44: mol_type = other DNA
gtcgtcctttggcccttccggtttagtggcccttccggtttagt

SEQ ID NO: 47 - DNA, 44 bp, synthetic construct
  source 1..44: mol_type = other DNA
ttccggggtttcaaacgccatatgtgtgcacctttcgatctacg

SEQ ID NO: 48 - DNA, 42 bp, synthetic construct
  source 1..42: mol_type = other DNA
tagatcgaaaggtgcacacatatggcgtttgaaaccccggaa

SEQ ID NO: 49 - DNA, 45 bp, synthetic construct
  source 1..45: mol_type = other DNA
cctcaatggctcttcctgtttagtttagcagtcgaagtacaattc

SEQ ID NO: 50 - DNA, 46 bp, synthetic construct
  source 1..46: mol_type = other DNA
tagatcgaaaggtgcacacatatgggttctaagtacacgagaaaag

SEQ ID NO: 51 - DNA, 37 bp, synthetic construct
  source 1..37: mol_type = other DNA
ctcttcctgtttagtttagtaaagggtaaggtactgc

SEQ ID NO: 52 - DNA, 46 bp, synthetic construct
  source 1..46: mol_type = other DNA
tagatcgaaaggtgcacacatatggcaaagtacactagagaagata

SEQ ID NO: 53 - DNA, 40 bp, synthetic construct
  source 1..40: mol_type = other DNA
ctcttcctgtttagtttaatactgagacatatactgttcg

SEQ ID NO: 54 - protein, 500 aa, synthetic construct
MSDSPKNAPRITDEADVVLIGAGIMSSTLGAMLRQLEPSWTQIVFERLDGPAQESSSPWNNAGTGHSALCELNYTPEVKGKVEIAKAVGINEKFQVSRQFWSHLVEEGVLSDPKEFINPVPHVSFGQGADQVAYIKARYEALKDHPLFQGMTYADDEATFTEKLPLMAKGRDFSDPVAISWIDEGTDINYGAQTKQYLDAAEVEGTEIRYGHEVKSIKADGAKWIVTVKNVHTGDTKTIKANFVFVGAGGYALDLLRSAGIPQVKGFAGFPVSGLWLRCTNEELIEQHAAKVYGKASVGAPPMSVPHLDTRVIEGEKGLLFGPYGGWTPKFLKEGSYLDLFKSIRPDNIPSYLGVAAQEFDLTKYLVTEVLKDQDKRMDALREYMPEAQNGDWETIVAGQRVQVIKPAGFPKFGSLEFGTTLINNSEGTIAGLLGASPGASIAPSAMIELLERCFGDRMIEWGDKLKDMIPSYGKKLASEPALFEQQWARTQKTLKLEEA

SEQ ID NO: 55 - DNA, 1503 bp, synthetic construct
  source 1..1503: mol_type = other DNA
atgtcagattccccgaagaacgcaccgaggattaccgatgaggcagatgtagttctcattggtgccggtatcatgagctccacgctgggtgcaatgctgcgtcagctggagccaagctggactcagatcgtcttcgagcgtttggatggaccggcacaagagtcgtcctccccgtggaacaatgcaggaaccggccactctgctctatgcgagctgaactacaccccagaggttaagggcaaggttgaaattgccaaggctgtaggaatcaacgagaagttccaggtttcccgtcagttctggtctcacctcgttgaagagggagtgctgtctgatcctaaggaattcatcaaccctgttcctcacgtatctttcggccagggcgcagatcaggttgcatacatcaaggctcgctacgaagctttgaaggatcacccactcttccagggcatgacctacgctgacgatgaagctaccttcaccgagaagctgcctttgatggcaaagggccgtgacttctctgatccagtagcaatctcttggatcgatgaaggcaccgacatcaactacggtgctcagaccaagcagtacctggatgcagctgaagttgaaggcactgaaatccgctatggccacgaagtcaagagcatcaaggctgatggcgcaaagtggatcgtgaccgtcaagaacgtacacactggcgacaccaagaccatcaaggcaaacttcgtgttcgtcggcgcaggcggatacgcactggatctgcttcgcagcgcaggcatcccacaggtcaagggcttcgctggattcccagtatccggcctgtggcttcgttgcaccaacgaggaactgatcgagcagcacgcagccaaggtatatggcaaggcatctgttggcgctcctccaatgtctgttcctcaccttgacacccgcgttatcgagggtgaaaagggtctgctctttggaccttacggtggctggacccctaagttcttgaaggaaggctcctacctggacctgttcaagtccatccgcccagacaacattccttcctaccttggcgttgctgctcaggaatttgatctgaccaagtaccttgtcactgaagttctcaaggaccaggacaagcgtatggatgctcttcgcgagtacatgccagaggcacaaaacggcgattgggagaccatcgttgccggacagcgtgttcaggttattaagcctgcaggattccctaagttcggttccctggaattcggcaccaccttgatcaacaactccgaaggcaccatcgccggattgctcggtgcttcccctggagcatccatcgcaccttccgcaatgatcgagctgcttgagcgttgcttcggtgaccgcatgatcgagtggggcgacaagctgaaggacatgatcccttcctacggcaagaagcttgcttccgagccagcactgtttgagcagcagtgggcacgcacccagaagaccctgaagcttgaggaagcctaa

SEQ ID NO: 56 - protein, 500 aa, synthetic construct
MSDSPKNAPRITDEADVVLIGAGIMSSTLGAMLRQLEPSWTQIVFERLDGPAQESSSPWNNAGTGHSALCELNYTPEVKGKVEIAKAVGINEKFQVSRQFWSHLVEEGVLADPKEFINPVPHVSFGQGADQVAYIKARYEALKDHPLFQGMTYADDEATFTEKLPLMAKGRDFSDPVAISWIDEGTDINYGAQTKQYLDASEVEGTEIRYGHEVKSIKADGAKWIVTVKNVHTGDTKTIKANFVFVGAGGYALDLLRSAGIPQVKGFAGFPVSGLWLRCTNEELIEQHAAKVYGKASVGAPPMSVPHLDTRVIEGEKGLLFGPYGGWTPKFLKEGSYLDLFKSIRPDNIPSYLGVAAQEFDLTKYLVTEVLKDQDKRMDALREYMPEAQNGDWETIVAGQRVQVIKPAGFPKFGSLEFGTTLINNSEGTIAGLLGASPGASIAPSAMIELLERCFGDRMIEWGDKLKDMIPSYGKKLASEPALFEQQWARTQKTLKLEEA

SEQ ID NO: 57 - DNA, 1503 bp, synthetic construct
  source 1..1503: mol_type = other DNA
atgtcagattccccgaagaacgcaccgaggattaccgatgaggcagatgtagttctcattggtgccggtatcatgagctccacgctgggtgcaatgctgcgtcagctggagccaagctggactcagatcgtcttcgagcgtttggatggaccggcacaagagtcgtcctccccgtggaacaatgcaggaaccggccactctgctctatgcgagctgaactacaccccagaggttaagggcaaggttgaaattgccaaggctgtaggaatcaacgagaagttccaggtttcccgtcagttctggtctcacctcgttgaagagggcgtgctggctgatcctaaggaattcatcaaccctgttcctcacgtatctttcggccagggcgcagaccaggttgcatacatcaaggctcgctacgaagctttgaaggatcacccactcttccagggcatgacctacgctgacgatgaagctaccttcaccgagaagctgcctttgatggcaaagggccgtgacttctctgatccagtagcaatctcttggatcgatgaaggcaccgacatcaactacggtgctcagaccaagcagtacctggatgcatctgaagttgaaggcactgaaatccgctatggccacgaagtcaagagcatcaaggctgatggcgcaaagtggatcgtgaccgtcaagaacgtacacactggcgacaccaagaccatcaaggcaaacttcgtgttcgtcggcgcaggcgggtacgcactggatctgcttcgcagcgcaggcatcccacaggtcaagggcttcgctggattcccagtatccggcctgtggcttcgttgcaccaacgaggaactgatcgagcagcacgcagccaaggtatatggcaaggcatctgttggcgctcctccaatgtctgttcctcaccttgacacccgcgttatcgagggtgaaaagggtctgctctttggaccttacggtggctggacccctaagttcttgaaggaaggctcctacctggacctgttcaagtccatccgcccagacaacattccttcctaccttggcgttgctgctcaggaatttgatctgaccaagtaccttgtcactgaagttctcaaggaccaggacaagcgtatggatgctcttcgcgagtacatgccagaggcacaaaacggcgattgggagaccatcgttgccggacagcgtgttcaggttattaagcctgcaggattccctaagttcggttccctggaattcggcaccaccttgatcaacaactccgaaggcaccatcgccggattgctcggtgcttcccctggagcatccatcgcaccttccgcaatgatcgagctgcttgagcgttgcttcggtgaccgcatgatcgagtggggcgacaagctgaaggacatgatcccttcctacggcaagaagcttgcttccgagccagcactgtttgagcagcagtgggcacgcacccagaagaccctgaagcttgaggaagcctaa

SEQ ID NO: 58 - protein, 328 aa, synthetic construct
MNSPQNVSTKKVTVTGAAGQISYSLLWRIANGEVFGTDTPVELKLLEIPQALGGAEGVAMELLDSAFPLLRNITITADANEAFDGANAAFLVGAKPRGKGEERADLLANNGKIFGPQGKAINDNAADDIRVLVVGNPANTNALIASAAAPDVPASRFNAMMRLDHNRAISQLATKLGRGSAEFNNIVVWGNHSATQFPDITYATVGGEKVTDLVDHDWYVEEFIPRVANRGAEIIEVRGKSSAASAASSAIDHMRDWVQGTEAWSSAAIPSTGAYGIPEGIFVGLPTVSRNGEWEIVEGLEISDFQRARIDANAQELQAEREAVRDLL

SEQ ID NO: 59 - DNA, 987 bp, synthetic construct
  source 1..987: mol_type = other DNA
atgaattccccgcagaacgtctccaccaagaaggtcaccgtcaccggcgcagctggtcaaatctcttattcactgttgtggcgcatcgccaacggtgaagtattcggcaccgacacccctgtagaactgaaacttctggagatccctcaggctcttggcggggcagagggtgtggctatggaacttctggattctgccttccccctcctgcgaaacatcaccatcaccgcggatgccaatgaggcattcgacggcgctaatgcggcgtttttggtcggtgcgaagcctcgcggaaaaggcgaagagcgcgcagatttgctggctaacaacggcaagattttcggacctcaaggtaaagctatcaatgacaacgccgcagatgacattcgtgtcctagttgttggaaacccagcgaacaccaacgcgttgattgcttcagctgcggccccagatgttccagcatcccgcttcaacgcaatgatgcgccttgatcacaaccgtgcgatctcccagctggccaccaagcttggccgtggatctgcggaatttaacaacattgtggtctggggaaatcactccgcaacccagttcccagacatcacctacgcaaccgttggtggagaaaaggtcactgacctggttgatcacgattggtatgtggaggagttcattcctcgcgtggctaaccgtggcgctgaaatcattgaggtccgtggaaagtcttctgcagcttctgcagcatcctctgcgattgatcacatgcgcgattgggtacagggcaccgaggcgtggtcctctgcggcaattccttccaccggtgcatacggcattcctgagggcatttttgtcggtctgccaaccgtatcccgcaacggtgagtgggaaatcgttgaaggcctggagatttccgatttccagcgcgcccgcatcgacgcgaatgctcaggaattgcaggccgagcgcgaggcagtgcgcgacttgctctaa

SEQ ID NO: 60 - protein, 426 aa, synthetic construct
MSSVSLQDFDAERIGLFHEDIKRKFDELKSKNLKLDLTRGKPSSEQLDFADELLALPGKGDFKAADGTDVRNYGGLDGIVDIRQIWADLLGVPVEQVLAGDASSLNIMFDVISWSYIFGNNDSVQPWSKEETVKWICPVPGYDRHFSITERFGFEMISVPMNEDGPDMDAVEELVKNPQVKGMWVVPVFSNPTGFTVTEDVAKRLSAMETAAPDFRVVWDNAYAVHTLTDEFPEVIDIVGLGEAAGNPNRFWAFTSTSKITLAGAGVSFFLTSAENRKWYTGHAGIRGIGPNKVNQLAHARYFGDAEGVRAVMRKHAASLAPKFNKVLEILDSRLAEYGVAQWTVPAGGYFISLDVVPGTASRVAELAKEAGIALTGAGSSYPLRQDPENKNLRLAPSLPPVEELEVAMDGVATCVLLAAAEHYAN

SEQ ID NO: 61 - DNA, 1281 bp, synthetic construct
  source 1..1281: mol_type = other DNA
atgagttcagtttcgctgcaggattttgatgcagagcgaattggtttgttccacgaggacattaagcgcaagtttgatgagctcaagtcaaaaaatctgaagctggatcttactcgcggtaagccttcgtcggagcagttggatttcgctgatgagttgttggcgttgcctggtaagggtgatttcaaggctgcggatggtactgatgtccgtaactatggcgggctggatggcatcgttgatattcgccagatttgggcggatttgctgggtgttcctgtggagcaggtcttggcgggggatgcttcgagcttgaacatcatgtttgatgtgatcagctggtcgtacattttcggtaacaatgattcggttcagccttggtcgaaggaagaaaccgttaagtggatttgccctgttccgggctatgatcgccatttctccatcacggagcgtttcggctttgagatgatttctgtgccaatgaatgaagacggccctgatatggatgctgttgaggaattggtgaagaatccgcaggttaagggcatgtgggttgttccggtgttttctaacccgactggtttcacggtgacagaagacgtcgcaaagcgtctaagcgcaatggaaaccgcagctccggacttccgcgttgtgtgggataatgcctacgccgttcatacgctgaccgatgaattccctgaggttatcgatatcgtcgggcttggtgaggccgctggcaacccgaaccgtttctgggcgttcacttctacttcgaagatcactctcgcgggtgcgggcgtgtcgttcttcctcacctctgcggagaaccgcaagtggtacaccggccatgcgggtatccgtggcattggccctaacaaggtcaatcagttggctcatgcgcgttactttggcgatgctgagggagtgcgcgcggtgatgcgtaagcatgctgcgtcgttggctccgaagttcaacaaggttctggagattctggattctcgccttgctgagtacggtgtcgcgcagtggactgtccctgcgggcggttacttcatttcccttgatgtggttcctggtacggcgtctcgcgtggctgagttggctaaggaagccggcatcgcgttgacgggtgcgggttcttcttacccgctgcgtcaggatccggagaacaaaaatctccgtttggcaccgtcgctgcctccagttgaggaacttgaggttgccatggatggcgtggctacctgtgtgctgttggcagcagcggagcattacgctaactaa

SEQ ID NO: 62 - protein, 447 aa, synthetic construct
MTVDEQVSNYYDMLLKRNAGEPEFHQAVAEVLESLKIVLEKDPHYADYGLIQRLCEPERQLIFRVPWVDDQGQVHVNRGFRVQFNSALGPYKGGLRFHPSVNLGIVKFLGFEQIFKNSLTGLPIGGGKGGSDFDPKGKSDLEIMRFCQSFMTELHRHIGEYRDVPAGDIGVGGREIGYLFGHYRRMANQHESGVLTGKGLTWGGSLVRTEATGYGCVYFVSEMIKAKGESISGQKIIVSGSGNVATYAIEKAQELGATVIGFSDSSGWVHTPNGVDVAKLREIKEVRRARVSVYADEVEGATYHTDGSIWDLKCDIALPCATQNELNGENAKTLADNGCRFVAEGANMPSTPEAVEVFRERDIRFGPGKAANAGGVATSALEMQQNASRDSWSFEYTDERLQVIMKNIFKTCAETAAEYGHENDYVVGANIAGFKKVADAMLAQGVI

SEQ ID NO: 63 - DNA, 1344 bp, synthetic construct
  source 1..1344: mol_type = other DNA
atgacagttgatgagcaggtctctaactattacgacatgcttctgaagcgcaatgctggcgagcctgaatttcaccaggcagtggcagaggttttggaatctttgaagatcgtcctggaaaaggaccctcattacgctgattacggtctcatccagcgcctgtgcgagcctgagcgtcagctcatcttccgtgtgccttgggttgatgaccagggccaggtccacgtcaaccgtggtttccgcgtgcagttcaactctgcacttggaccatacaagggcggcctgcgcttccacccatctgtaaacctgggcattgtgaagttcctgggctttgagcagatctttaaaaactccctaaccggcctgccaatcggtggtggcaagggtggatccgacttcgaccctaagggcaagtccgatctggaaatcatgcgtttctgccagtccttcatgaccgagctacaccgccacatcggtgagtaccgcgacgttcctgcaggtgacatcggagttggtggccgcgagatcggttacctgtttggccactaccgtcgcatggctaaccagcacgagtccggcgttttgaccggtaagggcctgacctggggtggatccctggtccgcaccgaggcaactggctacggctgcgtttacttcgtgagtgaaatgatcaaggctaagggcgagagcatcagcggccagaagatcatcgtttccggttccggcaacgtagcaacctacgcgattgaaaaggctcaggaactcggcgcaaccgttattggtttctccgattccagcggttgggttcatacccctaacggcgttgacgtggctaagctccgcgaaatcaaggaagttcgtcgcgcacgcgtatccgtgtacgccgacgaagttgaaggcgcaacctaccacaccgacggttccatctgggatctcaagtgcgatatcgctcttccttgtgcaactcagaacgagctcaacggcgagaacgctaagactcttgcagacaacggctgccgtttcgttgctgaaggcgcgaacatgccttccacccctgaggctgttgaggtcttccgtgagcgcgacatccgcttcggaccaggcaaggcagctaacgctggtggcgttgcaacctccgctctggagatgcagcagaacgcttcgcgcgattcctggagcttcgagtacaccgacgagcgcctccaggtgatcatgaagaacatcttcaagacctgtgcagagaccgcagcagagtatggacacgagaacgattacgttgtcggcgctaacattgctggcttcaagaaggtagctgacgcgatgctggcacagggcgtcatctaa

SEQ ID NO: 64 - protein, 469 aa, synthetic construct
MTEQEFRIEHDTMGEVKVPAKALWQAQTQRAVENFPISGRGLESAQIRAMGLLKAACAQVNKDSGALDAEKADAIIAAGKEIASGKHDAEFPIDVFQTGSGTSSNMNTNEVIASIAKANGVEVHPNDHVNMGQSSNDTFPTATHVAATEAAVNDLIPGLKVLHESLAKKANEWSEVVKSGRTHLMDAVPVTLGQEFGGYARQIQLGIERVEATLPRLGELAIGGTAAGTGINTSADFGGKVVAELINLTDVKELKEAENHFEAQAARDALVEFSGAMRVIAVSLYKIANDIRLMGSGPLTGLGEIRLPDLQPGSSIMPGKVNPVLCETATQVSAQVIGNDAAVAFSGTQGQFELNVFIPVMARNVLESARLLANTSRVFATRLVDGIEPNEAHMKELAESSPSIVTPLNSAIGYEAAAKVAKTALAEGKTIRQTVIDLGLVDGEKLTEEELDKRLDVLAMAHTERENKF

SEQ ID NO: 65 - DNA, 1410 bp, synthetic construct
  source 1..1410: mol_type = other DNA
atgaccgagcaggaattccgtattgagcacgacaccatgggtgaagtgaaggttccagcaaaggctctgtggcaggcacagacccagcgcgctgttgagaacttccctatctctggtcgtggtctggaatccgcacagatccgcgcaatgggtctgctgaaggcagcttgtgcgcaggtaaacaaggactccggtgcgctggatgcagagaaggcagatgccatcattgcagctggtaaggagatcgcgtccggtaagcatgacgctgagttcccaattgatgtgttccagactggttccggtacttcctccaacatgaacaccaatgaggttatcgcttccatcgcgaaggctaacggcgttgaggttcacccaaatgaccacgtcaacatgggtcagtcctccaatgacaccttccctactgcaactcacgttgctgcaaccgaagctgctgtcaatgacctcatcccaggcctgaaggttctgcacgagtctttggcgaagaaggctaacgagtggtctgaggttgttaagtccggccgcacccacctgatggacgctgttccagtaaccctgggccaggagttcggtggctacgctcgccagatccagctcggcatcgagcgcgttgaggctactcttcctcgccttggtgagctggctattggtggcaccgctgctggtaccggtatcaacacctccgctgatttcggcggcaaggttgttgctgaactgatcaacttgaccgacgtcaaggagctcaaggaagctgagaaccacttcgaggctcaggctgcacgcgacgctcttgttgagttctccggcgcaatgcgcgttatcgctgtctccttgtacaagatcgctaacgatatccgcctcatgggctccggcccactgaccggtcttggcgagatccgtctcccagacctgcagccaggttcctccatcatgccaggcaaggtcaacccagttctctgtgagaccgctacccaggtttccgctcaggttatcggcaatgacgcagctgttgcgttctccggcacccagggccagttcgagctcaacgtgttcatcccagtgatggctcgcaacgtgcttgagtccgctcgcctgctggctaacacttcccgcgtgttcgcaacccgtctcgttgatggcattgagccaaacgaggcacacatgaaggagctcgctgagtcttcaccttccatcgttaccccactgaactctgcaatcggctacgaagctgctgcaaaggtggctaagactgctttggctgagggcaagaccatccgccagactgtcatcgatttgggcttggttgatggcgagaagctcaccgaggaagagctggacaagcgcctcgacgttcttgctatggctcacaccgagcgcgagaacaagttctaa

SEQ ID NO: 66 - DNA, 42 bp, synthetic construct
  source 1..42: mol_type = other DNA
gtgaattcgagctcggtacccatactactcatgtttgcgaat

SEQ ID NO: 67 - DNA, 42 bp, synthetic construct
  source 1..42: mol_type = other DNA
tcctgatatcgggcaccatttggcaaagaatacgcaaagcac

SEQ ID NO: 68 - DNA, 41 bp, synthetic construct
  source 1..41: mol_type = other DNA
tgctttgcgtattctttgccaaatggtgcccgatatcagga

SEQ ID NO: 69 - DNA, 42 bp, synthetic construct
  source 1..42: mol_type = other DNA
aacaaagcagccatgcgttgcagccgttacttaaaccaagtc

SEQ ID NO: 70 - DNA, 43 bp, synthetic construct
  source 1..43: mol_type = other DNA
cgacttggtttaagtaacggctgcaacgcatggctgctttgtt

SEQ ID NO: 71 - DNA, 42 bp, synthetic construct
  source 1..42: mol_type = other DNA
gcgaatgagaccagttgactgttagttagcgtaatgctccgc

SEQ ID NO: 72 - DNA, 42 bp, synthetic construct
  source 1..42: mol_type = other DNA
gcggagcattacgctaactaacagtcaactggtctcattcgc

SEQ ID NO: 73 - DNA, 42 bp, synthetic construct
  source 1..42: mol_type = other DNA
ggttaatatccaatatggaagttagatgacgccctgtgccag

SEQ ID NO: 74 - DNA, 42 bp, synthetic construct
  source 1..42: mol_type = other DNA
ctggcacagggcgtcatctaacttccatattggatattaacc

SEQ ID NO: 75 - DNA, 42 bp, synthetic construct
  source 1..42: mol_type = other DNA
attcgcaaacatgagtagtatttagaacttgttctcgcgctc

SEQ ID NO: 76 - DNA, 41 bp, synthetic construct
  source 1..41: mol_type = other DNA
cgcgagaacaagttctaaatactactcatgtttgcgaattg

SEQ ID NO: 77 - DNA, 42 bp, synthetic construct
  source 1..42: mol_type = other DNA
ggtcgactctagaggatccccttaggcttcctcaagcttcag

SEQ ID NO: 78 - DNA, 15 bp, synthetic construct
  source 1..15: mol_type = other DNA
ctcttcaccagcatt

SEQ ID NO: 79 - DNA, 20 bp, synthetic construct
  source 1..20: mol_type = other DNA
ttgtcacaacatctgtttca

SEQ ID NO: 80 - DNA, 5802 bp, synthetic construct
  source 1..5802: mol_type = other DNA
gttcgcttgctgtccataaaaccgcccagtctagctatcgccatgtaagcccactgcaagctacctgctttctctttgcgcttgcgttttcccttgtccagatagcccagtagctgacattcatccggggtcagcaccgtttctgcggactggctttctacgtgttccgcttcctttagcagcccttgcgccctgagtgcttgcggcagcgtgaagctagcttttatcgccattcgccattcaggctgcgcaactgttgggaagggcgatcggtgcgggcctcttcgctattacgccagctggcgaaagggggatgtgctgcaaggcgattaagttgggtaacgccagggttttcccagtcacgacgttgtaaaacgacggccagtgaattcgagctcggtacccggggatcctctagagtcgacctgcaggcatgcaagcttggcgtaatcatggtcatagctgtttcctgtgtgaaattgttatccgctcacaattccacacaacatacgagccggaagcataaagtgtaaagcctggggtgcctaatgagtgagctaactcacattaattgcgttgcgctcactgcccgctttccagtcgggaaacctgtcgtgccagctgcattaatgaatcggccaacgcgcggggagaggcggtttgcgtattgggcgctcttccgcttcctcgctcactgactcgctgcgctcggtcgttcggctgcggcgagcggtatcagctcactcaaaggcggtaatacggttatccacagaatcaggggataacgcaggaaagaacatgtgagcaaaaggccagcaaaaggccaggaaccgtaaaaaggccgcgttgctggcgtttttccataggctccgcccccctgacgagcatcacaaaaatcgacgctcaagtcagaggtggcgaaacccgacaggactataaagataccaggcgtttccccctggaagctccctcgtgcgctctcctgttccgaccctgccgcttaccggatacctgtccgcctttctcccttcgggaagcgtggcgctttctcaatgctcacgctgtaggtatctcagttcggtgtaggtcgttcgctccaagctgggctgtgtgcacgaaccccccgttcagcccgaccgctgcgccttatccggtaactatcgtcttgagtccaacccggtaagacacgacttatcgccactggcagcagccactggtaacaggattagcagagcgaggtatgtaggcggtgctacagagttcttgaagtggtggcctaactacggctacactagaaggacagtatttggtatctgcgctctgctgaagccagttaccttcggaaaaagagttggtagctcttgatccggcaaacaaaccaccgctggtagcggtggtttttttgtttgcaagcagcagattacgcgcagaaaaaaaggatctcaagaagatcctttgatcttttctacggggtctgacgctcagtggaacgaaaactcacgttaagggattttggtcatgagattatcaaaaaggatcttcacctagatccttttggggtgggcgaagaactccagcatgagatccccgcgctggaggatcatccagccctgatagaaacagaagccactggagcacctcaaaaacaccatcatacactaaatcagtaagttggcagcatcacccgacgcactttgcgccgaataaatacctgtgacggaagatcacttcgcagaataaataaatcctggtgtccctgttgataccgggaagccctgggccaacttttggcgaaaatgagacgttgatcggcacgtaagaggttccaactttcaccataatgaaataagatcactaccgggcgtattttttgagttatcgagattttcaggagctgatagaaacagaagccactggagcacctcaaaaacaccatcatacactaaatcagtaagttggcagcatcacccgacgcactttgcgccgaataaatacctgtgacggaagatcacttcgcagaataaataaatcctggtgtccctgttgataccgggaagccctgggccaacttttggcgaaaatgagacgttgatcggcacgtaagaggttccaactttcaccataatgaaataagatcactaccgggcgtattttttgagttatcgagattttcaggagctctttggcatcgtctctcgcctgtcccctcagttcagtaatttcctgcatttgcctgtttccagtcggtagatattccacaaaacagcagggaagcagcgcttttccgctgcataaccctgcttcggggtcattatagcgattttttcggtatatccatcctttttcgcacgatatacaggattttgccaaagggttcgtgtagactttccttggtgtatccaacggcgtcagccgggcaggataggtgaagtaggcccacccgcgagcgggtgttccttcttcactgtcccttattcgcacctggcggtgctcaacgggaatcctgctctgcgaggctggccggctaccgccggcgtaacagatgagggcaagcggatggctgatgaaaccaagccaaccaggaagggcagcccacctatcaaggtgtactgccttccagacgaacgaagagcgattgaggaaaaggcggcggcggccggcatgagcctgtcggcctacctgctggccgtcggccagggctacaaaatcacgggcgtcgtggactatgagcacgtccgcgagggcgtcccggaaaacgattccgaagcccaacctttcatagaaggcggcggtggaatcgaaatctcgtgatggcaggttgggcgtcgcttggtcggtcatttcgaaaaaggttaggaatacggttagccatttgcctgcttttatatagttcatatgggattcacctttatgttgataagaaataaaagaaaatgccaataggatatcggcattttcttttgcgtttttatttgttaactgttaattgtccttgttcaaggatgctgtctttgacaacagatgttttcttgcctttgatgttcagcaggaagctcggcgcaaacgttgattgtttgtctgcgtagaatcctctgtttgtcatatagcttgtaatcacgacattgtttcctttcgcttgaggtacagcgaagtgtgagtaagtaaaggttacatcgttaggcggatcaagatccatttttaacacaaggccagttttgttcagcggcttgtatgggccagttaaagaattagaaacataaccaagcatgtaaatatcgttagacgtaatgccgtcaatcgtcatttttgatccgcgggagtcagtgaacaggtaccatttgccgttcattttaaagacgttcgcgcgttcaatttcatctgttactgtgttagatgcaatcagcggtttcatcacttttttcagtgtgtaatcatcgtttagctcaatcataccgagagcgccgtttgctaactcagccgtgcgttttttatcgctttgcagaagtttttgactttcttgacggaagaatgatgtgcttttgccatagtatgctttgttaaataaagattcttcgccttggtagccatcttcagttccagtgtttgcttcaaatactaagtatttgtggcctttatcttctacgtagtgaggatctctcagcgtatggttgtcgcctgagctgtagttgccttcatcgatgaactgctgtacattttgatacgtttttccgtcaccgtcaaagattgatttataatcctctacaccgttgatgttcaaagagctgtctgatgctgatacgttaacttgtgcagttgtcagtgtttgtttgccgtaatgtttaccggagaaatcagtgtagaataaacggatttttccgtcagatgtaaatgtggctgaacctgaccattcttgtgtttggtcttttaggatagaatcatttgcatcgaatttgtcgctgtctttaaagacgcggccagcgtttttccagctgtcaatagaagtttcgccgactttttgatagaacatgtaaatcgatgtgtcatccgcatttttaggatctccggctaatgcaaagacgatgtggtagccgtgatagtttgcgacagtgccgtcagcgttttgtaatggccagctgtcccaaacgtccaggccttttgcagaagagatatttttaattgtggacgaatcaaattcagaaacttgatatttttcatttttttgctgttcagggatttgcagcatatcatggcgtgtaatatgggaaatgccgtatgtttccttatatggcttttggttcgtttctttcgcaaacgcttgagttgcgcctcctgccagcagtgcggtagtaaaggttaatactgttgcttgttttgcaaactttttgatgttcatcgttcatgtctccttttttatgtactgtgttagcggtctgcttcttccagccctcctgtttgaagatggcaagttagttacgcacaataaaaaaagacctaaaatatgtaaggggtgacgccaaagtatacactttgccctttacacattttaggtcttgcctgctttatcagtaacaaacccgcgcgatttacttttcgacctcattctattagactctcgtttggattgcaactggtctattttcctcttttgtttgatagaaaatcataaaaggatttgcagactacgggcctaaagaactaaaaaatctatctgtttcttttcattctctgtattttttatagtttctgttgcatgggcataaagttgcctttttaatcacaattcagaaaatatcataatatctcatttcactaaataatagtgaacggcaggtatatgtgatgggttaaaaaggatcaccccagagtcccgctcagaagaactcgtcaagaaggcgatagaaggcgatgcgctgcgaatcgggagcggcgataccgtaaagcacgaggaagcggtcagcccattcgccgccaagctcttcagcaatatcacgggtagccaacgctatgtcctgatagcggtccgccacacccagccggccacagtcgatgaatccagaaaagcggccattttccaccatgatattcggcaagcaggcatcgccatgggtcacgacgagatcctcgccgtcgggcatccgcgccttgagcctggcgaacagttcggctggcgcgagcccctgatgctcttcgtccagatcatcctgatcgacaagaccggcttccatccgagtacgtgctcgctcgatgcgatgtttcgcttggtggtcgaatgggcaggtagccggatcaagcgtatgcagccgccgcattgcatcagccatgatggatactttctcggcaggagcaaggtgagatgacaggagatcctgccccggcacttcgcccaatagcagccagtcccttcccgcttcagtgacaacgtcgagacagctgcgcaaggaacgcccgtcgtggccagccacgatagccgcgctgcctcgtcttggagttcattcagggcaccggacaggtcggtcttgacaaaaagaaccgggcgcccctgcgctgacagccggaacacggcggcatcagagcagccgattgtctgttgtgcccagtcatagccgaatagcctctccacccaagcggccggagaacctgcgtgcaatccatcttgttcaatcatgcgaaacgatcctcatcctgtctcttgatcagatcttgatcccctgcgccatcagatccttggcggcaagaaagccatccagtttactttgcagggcttcccaaccttaccagagggcgccccagctggcaattccg